European Patent Application EP 4 685 156 A2, published January 28, 2026. Title: Process for preparing a GIP/GLP1 dual agonist. Applicant: Eli Lilly and Company. The sequence listing filed with the application follows.

SEQUENCE LISTING (40 sequences)

SEQ ID NO: 1 - protein, 39 aa, synthetic construct
  REGION 1..39: note = Synthetic Construct
  SITE 2: note = MISC_FEATURE - Xaa at position 2 is nonnaturally occurring amino acid 2-Aminoisobutyric Acid
  SITE 13: note = MISC_FEATURE - Xaa at position 13 is nonnaturally occurring amino acid 2-Aminoisobutyric Acid
  MOD_RES 20: note = Lys at position 20 is chemically modified through conjugation to the epsilon-amino group of the K side-chain with (2-[2-(2-Amino-ethoxy)-ethoxy]-acetyl)2-(gamma-Glu)1-CO-(CH2)18-C O2H
  MOD_RES 39: note = Ser at position 39 is amidated as a C-terminal primary amide
YXEGTFTSDYSIXLDKIAQKAFVQWLIAGGPSSGAPPPS

SEQ ID NO: 2 - protein, 10 aa, synthetic construct
  REGION 1..10: note = Synthetic Construct
  MOD_RES 3: note = The sidechain of serine is protected by t-butyl.
  MOD_RES 4: note = The sidechain of serine is protected by t-butyl.
  MOD_RES 10: note = The sidechain of serine is protected by t-butyl.
  MOD_RES 10: note = Serine at position 10 is amidated as a C-terminal primary amide.
GPSSGAPPPS

SEQ ID NO: 3 - protein, 15 aa, synthetic construct
  REGION 1..15: note = Synthetic Construct
  MOD_RES 1: note = N-terminus is protected by Fmoc.
  MOD_RES 1: note = The sidechain of aspartic acid is protected by t-butyl.
  MOD_RES 2: note = The sidechain of lysine is protected by a t-butyloxycarbonyl (Boc) protecting group.
  MOD_RES 5: note = The sidechain of glutamine is protected by a Trityl (Trt) protecting group.
  MOD_RES 6: note = The epsilon amino group of K is modified with -CO-O-CH2-CH=CH2
  MOD_RES 10: note = The sidechain of glutamine is protected by a Trityl (Trt) protecting group.
  MOD_RES 11: note = The sidechain of Tryptophan is protected by a t-butyloxycarbonyl (Boc) protecting group.
DKIAQKAFVQWLIAG

SEQ ID NO: 4 - protein, 14 aa, synthetic construct
  REGION 1..14: note = Synthetic Construct
  MOD_RES 1: note = N-terminus is protected by (t-butyloxycarbonyl) Boc.
  MOD_RES 1: note = The sidechain of tyrosine is protected by t-butyl.
  MOD_RES 2: note = Xaa at position 2 is 2-Aminoisobutyric Acid (Aib).
  MOD_RES 3: note = The sidechain of glutamic acid is protected with t-Butyl.
  MOD_RES 5: note = The sidechain of threonine is protected with t-Butyl.
  MOD_RES 7: note = The sidechain of threonine is protected with t-Butyl.
  MOD_RES 8: note = The sidechain of serine is protected with t-Butyl.
  MOD_RES 9: note = The sidechain of aspartic acid is protected with t-Butyl.
  MOD_RES 10: note = The sidechain of tyrosine is protected with t-Butyl.
  MOD_RES 11: note = The sidechain of serine is protected with t-Butyl.
  MOD_RES 13: note = Xaa at position 13 is 2-Aminoisobutyric Acid (Aib).
YXEGTFTSDYSIXL

SEQ ID NO: 5 - protein, 25 aa, synthetic construct
  REGION 1..25: note = Synthetic Construct
  MOD_RES 1: note = The sidechain of aspartic acid is protected by t-butyl.
  MOD_RES 2: note = The sidechain of lysine is protected by a t-butyloxycarbonyl (Boc) protecting group.
  MOD_RES 5: note = The sidechain of glutamine is protected by a Trityl (Trt) protecting group.
  MOD_RES 6: note = The lysine at position 6 is chemically modified through conjugation to the epsilon-amino group of the K side-chain with C(O)-O-CH2-CH=CH2.
  MOD_RES 10: note = The sidechain of glutamine is protected by a Trityl (Trt) protecting group.
  MOD_RES 11: note = The sidechain of tryptophan is protected by Boc.
  MOD_RES 18: note = The sidechain od serine is protected by t-butyl.
  MOD_RES 19: note = The sidechain of serine is protected by t-butyl.
  MOD_RES 25: note = The sidechain of serine is protected by t-butyl.
  MOD_RES 25: note = Serine at position 25 is amidated as a C-terminal primary amide.
DKIAQKAFVQWLIAGGPSSGAPPPS

SEQ ID NO: 6 - protein, 39 aa, synthetic construct; identical to SEQ ID NO: 1
  REGION 1..39: note = Synthetic Construct
  MOD_RES 1: note = N-terminus is protected by (t-butyloxycarbonyl) Boc.
  MOD_RES 1: note = The sidechain of tyrosine is protected by t-butyl.
  MOD_RES 2: note = Xaa at position 2 is 2-Aminoisobutyric Acid (Aib).
  MOD_RES 3: note = The sidechain of glutamic acid is protected by t-butyl.
  MOD_RES 5: note = The sidechain of threoinine is protected by t-butyl.
  MOD_RES 7: note = The sidechain of threoinine is protected by t-butyl.
  MOD_RES 8: note = The sidechain of serine is protected by t-butyl.
  MOD_RES 9: note = The sidechain of aspartic acic is protected by t-butyl.
  MOD_RES 10: note = The sidechain of tyrosine is protected by t-butyl.
  MOD_RES 11: note = The sidechain of serine is protected by t-butyl.
  MOD_RES 13: note = Xaa at position 13 is 2-Aminoisobutyric Acid (Aib).
  MOD_RES 15: note = The sidechain of aspartic acid is protected by t-butyl.
  MOD_RES 16: note = The sidechain of lysine is protected by a t-butyloxycarbonyl (Boc) protecting group.
  MOD_RES 19: note = The sidechain of glutamine is protected by a Trityl (Trt) protecting group.
  MOD_RES 20: note = The lysine at position 6 is chemically modified through conjugation to the epsilon-amino group of the K side-chain with C(O)-O-CH2-CH=CH2.
  MOD_RES 24: note = The sidechain of glutamine is protected by a Trityl (Trt) protecting group.
  MOD_RES 25: note = The sidechain of Tryptophan is protected by a t-butyloxycarbonyl (Boc) protecting group.
  MOD_RES 32: note = The sidechain of serine is protected by t-butyl.
  MOD_RES 33: note = The sidechain of serine is protected by t-butyl.
  MOD_RES 39: note = The sidechain of serine is protected by t-butyl.
  MOD_RES 39: note = Serine at position 39 is amidated as a C-terminal primary amide.

SEQ ID NO: 7 - protein, 39 aa, synthetic construct; identical to SEQ ID NO: 1
  REGION 1..39: note = Synthetic Construct
  MOD_RES 1: note = N-terminus is protected by (t-butyloxycarbonyl) Boc.
  MOD_RES 1: note = The sidechain of tyrosine is protected by t-butyl.
  MOD_RES 2: note = Xaa at position 2 is 2-Aminoisobutyric Acid (Aib).
  MOD_RES 3: note = The sidechain of glutamic acid is protected by t-butyl.
  MOD_RES 5: note = The sidechain of threonine is protected by t-butyl.
  MOD_RES 7: note = The sidechain of threonine is protected by t-butyl.
  MOD_RES 8: note = The sidechain of serine is protected by t-butyl.
  MOD_RES 9: note = The sidechain of aspartic acid is protected by t-butyl.
  MOD_RES 10: note = The sidechain of tyrosine is protected by t-butyl.
  MOD_RES 11: note = The sidechain of serine is protected by t-butyl.
  MOD_RES 13: note = Xaa at position 13 is 2-Aminoisobutyric Acid (Aib).
  MOD_RES 15: note = The sidechain of aspartic acid is protected by t-butyl.
  MOD_RES 16: note = The sidechain of lysine is protected by a t-butyloxycarbonyl (Boc) protecting group.
  MOD_RES 19: note = The sidechain of glutamine is protected by a Trityl (Trt) protecting group.
  MOD_RES 24: note = The sidechain of glutamine is protected by a Trityl (Trt) protecting group.
  MOD_RES 25: note = The sidechain of Tryptophan is protected by a t-butyloxycarbonyl (Boc) protecting group.
  MOD_RES 32: note = The sidechain of serine is protected by t-butyl.
  MOD_RES 33: note = The sidechain of serine is protected by t-butyl.
  MOD_RES 39: note = The sidechain of serine is protected by t-butyl.
  MOD_RES 39: note = Serine at position 39 is amidated as a C-terminal primary amide.

SEQ ID NO: 8 - protein, 39 aa, synthetic construct; identical to SEQ ID NO: 1
  REGION 1..39: note = Synthetic Construct
  MOD_RES 1: note = N-terminus is protected by (t-butyloxycarbonyl) Boc.
  MOD_RES 1: note = The sidechain of tyrosine is protected by t-butyl.
  MOD_RES 2: note = Xaa at position 2 is 2-Aminoisobutyric Acid (Aib).
  MOD_RES 3: note = The sidechain of glutamic acid is protected by t-butyl.
  MOD_RES 5: note = The sidechain of threonine is protected by t-butyl.
  MOD_RES 7: note = The sidechain of threonine is protected by t-butyl.
  MOD_RES 8: note = The sidechain of serine is protected by t-butyl.
  MOD_RES 9: note = The sidechain of aspartic acid is protected by t-butyl.
  MOD_RES 10: note = The sidechain of tyrosine is protected by t-butyl.
  MOD_RES 11: note = The sidechain of serine is protected by t-butyl.
  MOD_RES 13: note = Xaa at position 13 is 2-Aminoisobutyric Acid (Aib).
  MOD_RES 15: note = The sidechain of aspartic acid is protected by t-butyl.
  MOD_RES 16: note = The sidechain of lysine is protected by a t-butyloxycarbonyl (Boc) protecting group.
  MOD_RES 19: note = The sidechain of glutamine is protected by a Trityl (Trt) protecting group.
  MOD_RES 20: note = Lys at position 20 is chemically modified through conjugation to the epsilon-amino group of the K side-chain with (2-[2-(2-Amino-ethoxy)-ethoxy]-acetyl)2-(gamma-Glu(t-butyl))1-CO- (CH2)18-CO2-(t-butyl).
  MOD_RES 24: note = The sidechain of glutamine is protected by a Trityl (Trt) protecting group.
  MOD_RES 25: note = The sidechain of Tryptophan is protected by a t-butyloxycarbonyl (Boc) protecting group.
  MOD_RES 32: note = The sidechain of serine is protected by t-butyl.
  MOD_RES 33: note = The sidechain of serine is protected by t-butyl.
  MOD_RES 39: note = The sidechain of serine is protected by t-butyl.
  MOD_RES 39: note = Serine at position 39 is amidated as a C-terminal primary amide.

SEQ ID NO: 9 - protein, 9 aa, synthetic construct
  REGION 1..9: note = Synthetic Construct
  MOD_RES 1: note = N-terminus is protected by Fmoc.
  MOD_RES 2: note = The sidechain of serine is protected by t-butyl.
  MOD_RES 3: note = The sidechain of serine is protected by t-butyl.
  MOD_RES 9: note = The sidechain of serine is protected by t-butyl.
  MOD_RES 9: note = Serine at position 9 is amidated as a C-terminal primary amide.
PSSGAPPPS

SEQ ID NO: 10 - protein, 9 aa, synthetic construct
  REGION 1..9: note = Synthetic Construct
  MOD_RES 1: note = N-terminus is protected by Fmoc.
  MOD_RES 3: note = The sidechain of glutamine is protected by a Trityl (Trt) protecting group.
  MOD_RES 4: note = The sidechain of Tryptophan is protected by a t-butyloxycarbonyl (Boc) protecting group.
FVQWLIAGG

SEQ ID NO: 11 - protein, 8 aa, synthetic construct
  REGION 1..8: note = Synthetic Construct
  MOD_RES 1: note = N-terminus is protected by Fmoc.
  MOD_RES 2: note = The sidechain of aspartic acid is protected by t-butyl.
  MOD_RES 3: note = The sidechain of lysine is protected by a t-butyloxycarbonyl (Boc) protecting group.
  MOD_RES 6: note = The sidechain of glutamine is protected by a Trityl (Trt) protecting group.
  MOD_RES 7: note = Lys at position 7 is chemically modified through conjugation to the epsilon-amino group of the K side-chain with (2-[2-(2-Amino-ethoxy)-ethoxy]-acetyl)2-(gamma-Glu(t-butyl))1-CO- (CH2)18-CO2-(t-butyl).
LDKIAQKA

SEQ ID NO: 12 - protein, 13 aa, synthetic construct
  REGION 1..13: note = Synthetic Construct
  MOD_RES 1: note = N-terminus is protected by (t-butyloxycarbonyl) Boc.
  MOD_RES 1: note = The sidechain of tyrosine is protected by t-butyl.
  MOD_RES 2: note = Xaa at position 2 is 2-Aminoisobutyric Acid (Aib).
  MOD_RES 3: note = The sidechain of glutamic acid is protected by t-butyl.
  MOD_RES 5: note = The sidechain of threonine is protected by t-butyl.
  MOD_RES 7: note = The sidechain of threonine is protected by t-butyl.
  MOD_RES 8: note = The sidechain of serine is protected by t-butyl.
  MOD_RES 9: note = The sidechain of aspartic acid is protected by t-butyl.
  MOD_RES 10: note = The sidechain of tyrosine is protected by t-butyl.
  MOD_RES 11: note = The sidechain of serine is protected by t-butyl.
  MOD_RES 13: note = Xaa at position 13 is 2-Aminoisobutyric Acid (Aib).
YXEGTFTSDYSIX

SEQ ID NO: 13 - protein, 18 aa, synthetic construct
  REGION 1..18: note = Synthetic Construct
  MOD_RES 3: note = The sidechain of glutamine is protected by a Trityl (Trt) protecting group.
  MOD_RES 4: note = The sidechain of Tryptophan is protected by a t-butyloxycarbonyl (Boc) protecting group.
  MOD_RES 11: note = The sidechain of serine is protected by t-butyl.
  MOD_RES 12: note = The sidechain of serine is protected by t-butyl.
  MOD_RES 18: note = The sidechain of serine is protected by t-butyl.
  MOD_RES 18: note = Serine at position 18 is amidated as a C-terminal primary amide.
FVQWLIAGGPSSGAPPPS

SEQ ID NO: 14 - protein, 26 aa, synthetic construct
  REGION 1..26: note = Synthetic Construct
  MOD_RES 2: note = The sidechain of aspartic acid is protected by t-butyl.
  MOD_RES 3: note = The sidechain of lysine is protected by a t-butyloxycarbonyl (Boc) protecting group.
  MOD_RES 6: note = The sidechain of glutamine is protected by a Trityl (Trt) protecting group.
  MOD_RES 7: note = Lys at position 7 is chemically modified through conjugation to the epsilon-amino group of the K side-chain with (2-[2-(2-Amino-ethoxy)-ethoxy]-acetyl)2-(gamma-Glu(t-butyl))1-CO- (CH2)18-CO2-(t-butyl).
  MOD_RES 11: note = The sidechain of glutamine is protected by a Trityl (Trt) protecting group.
  MOD_RES 12: note = The sidechain of Tryptophan is protected by a t-butyloxycarbonyl (Boc) protecting group.
  MOD_RES 19: note = The sidechain of serine is protected by t-butyl.
  MOD_RES 20: note = The sidechain of serine is protected by t-butyl.
  MOD_RES 26: note = The sidechain of serine is protected by t-butyl.
  MOD_RES 26: note = Serine at position 26 is amidated as a C-terminal primary amide.
LDKIAQKAFVQWLIAGGPSSGAPPPS

SEQ ID NO: 15 - protein, 39 aa, synthetic construct; identical to SEQ ID NO: 1
  REGION 1..39: note = Synthetic Construct
  MOD_RES 1: note = N-terminus is protected by (t-butyloxycarbonyl) Boc.
  MOD_RES 1: note = The sidechain of tyrosine is protected by t-butyl.
  MOD_RES 2: note = Xaa at position 2 is 2-Aminoisobutyric Acid (Aib).
  MOD_RES 3: note = The sidechain of glutamic acid is protected by t-butyl.
  MOD_RES 5: note = The sidechain of threonine is protected by t-butyl.
  MOD_RES 7: note = The sidechain of threonine is protected by t-butyl.
  MOD_RES 8: note = The sidechain of serine is protected by t-butyl.
  MOD_RES 9: note = The sidechain of aspartic acid is protected by t-butyl.
  MOD_RES 10: note = The sidechain of tyrosine is protected by t-butyl.
  MOD_RES 11: note = The sidechain of serine is protected by t-butyl.
  MOD_RES 13: note = Xaa at position 13 is 2-Aminoisobutyric Acid (Aib).
  MOD_RES 15: note = The sidechain of aspartic acid is protected by t-butyl.
  MOD_RES 16: note = The sidechain of lysine is protected by a t-butyloxycarbonyl (Boc) protecting group.
  MOD_RES 19: note = The sidechain of glutamine is protected by a Trityl (Trt) protecting group.
  MOD_RES 20: note = Lys at position 20 is chemically modified through conjugation to the epsilon-amino group of the K side-chain with (2-[2-(2-Amino-ethoxy)-ethoxy]-acetyl)2-(gamma-Glu(t-butyl))1-CO- (CH2)18-CO2-(t-butyl).
  MOD_RES 24: note = The sidechain of glutamine is protected by a Trityl (Trt) protecting group.
  MOD_RES 25: note = The sidechain of Tryptophan is protected by a t-butyloxycarbonyl (Boc) protecting group.
  MOD_RES 32: note = The sidechain of serine is protected by t-butyl.
  MOD_RES 33: note = The sidechain of serine is protected by t-butyl.
  MOD_RES 39: note = The sidechain of serine is protected by t-butyl.
  MOD_RES 39: note = Serine at position 39 is amidated as a C-terminal primary amide.

SEQ ID NO: 16 - protein, 8 aa, synthetic construct
  REGION 1..8: note = Synthetic Construct
  MOD_RES 1: note = N-terminus is protected by Fmoc.
  MOD_RES 3: note = The sidechain of glutamine is protected by a Trityl (Trt) protecting group.
  MOD_RES 4: note = The sidechain of Tryptophan is protected by a t-butyloxycarbonyl (Boc) protecting group.
FVQWLIAG

SEQ ID NO: 17 - protein, 7 aa, synthetic construct
  REGION 1..7: note = Synthetic Construct
  MOD_RES 1: note = N-terminus is protected by Fmoc.
  MOD_RES 1: note = The sidechain of aspartic acid is protected by t-butyl.
  MOD_RES 2: note = The sidechain of lysine is protected by a t-butyloxycarbonyl (Boc) protecting group.
  MOD_RES 5: note = The sidechain of glutamine is protected by a Trityl (Trt) protecting group.
  MOD_RES 6: note = Lys at position 6 is chemically modified through conjugation to the epsilon-amino group of the K side-chain with (2-[2-(2-Amino-ethoxy)-ethoxy]-acetyl)2-(gamma-Glu(t-butyl))1-CO- (CH2)18-CO2-(t-butyl).
DKIAQKA

SEQ ID NO: 18 - protein, 14 aa, synthetic construct
  REGION 1..14: note = Synthetic Construct
  MOD_RES 1: note = N-terminus is protected by (t-butyloxycarbonyl) Boc.
  MOD_RES 1: note = The sidechain of tyrosine is protected by t-butyl.
  MOD_RES 2: note = Xaa at position 2 is 2-Aminoisobutyric Acid (Aib).
  MOD_RES 3: note = The sidechain of glutamic acid is protected by t-butyl.
  MOD_RES 5: note = The glycine at position 4 combines with position 5 to create Gly-Thr (psiMe,Me-Pro) using pseudoproline.
  MOD_RES 7: note = The sidechain of threonine is protected by t-butyl.
  MOD_RES 8: note = The sidechain of serine is protected by t-butyl.
  MOD_RES 9: note = The sidechain of aspartic acid is protected by t-butyl.
  MOD_RES 10: note = The sidechain of tyrosine is protected by t-butyl.
  MOD_RES 11: note = The sidechain of serine is protected by t-butyl.
  MOD_RES 13: note = Xaa at position 13 is 2-Aminoisobutyric Acid (Aib).
YXEGXFTSDYSIXL

SEQ ID NO: 19 - protein, 14 aa, synthetic construct
  REGION 1..14: note = Synthetic Construct
  MOD_RES 1: note = N-terminus is protected by (t-butyloxycarbonyl) Boc.
  MOD_RES 1: note = The sidechain of tyrosine is protected by t-butyl.
  MOD_RES 2: note = Xaa at position 2 is 2-Aminoisobutyric Acid (Aib).
  MOD_RES 3: note = The sidechain of glutamic acid is protected by t-butyl.
  MOD_RES 5: note = The sidechain of threonine is protected by t-butyl.
  MOD_RES 7: note = The sidechain of threonine is protected by t-butyl.
  MOD_RES 8: note = The sidechain of serine is protected by t-butyl.
  MOD_RES 9: note = The sidechain of aspartic acid is protected by t-butyl.
  MOD_RES 10: note = The sidechain of tyrosine is protected by t-butyl.
  MOD_RES 11: note = The sidechain of serine is protected by t-butyl.
  MOD_RES 13: note = Xaa at position 13 is 2-Aminoisobutyric Acid (Aib).
YXEGTFTSDYSIXL

SEQ ID NO: 20 - protein, 18 aa, synthetic construct
  REGION 1..18: note = Synthetic Construct
  MOD_RES 3: note = The sidechain of glutamine is protected by a Trityl (Trt) protecting group.
  MOD_RES 4: note = The sidechain of Tryptophan is protected by a t-butyloxycarbonyl (Boc) protecting group.
  MOD_RES 11: note = The sidechain of serine is protected by t-butyl.
  MOD_RES 12: note = The sidechain of serine is protected by t-butyl.
  MOD_RES 18: note = The sidechain of serine is protected by t-butyl.
  MOD_RES 18: note = Serine at position 18 is amidated as a C-terminal primary amide.
FVQWLIAGGPSSGAPPPS

SEQ ID NO: 21 - protein, 25 aa, synthetic construct
  REGION 1..25: note = Synthetic Construct
  MOD_RES 1: note = The sidechain of aspartic acid is protected by t-butyl.
  MOD_RES 2: note = The sidechain of lysine is protected by a t-butyloxycarbonyl (Boc) protecting group.
  MOD_RES 5: note = The sidechain of glutamine is protected by a Trityl (Trt) protecting group.
  MOD_RES 6: note = Lys at position 6 is chemically modified through conjugation to the epsilon-amino group of the K side-chain with (2-[2-(2-Amino-ethoxy)-ethoxy]-acetyl)2-(gamma-Glu(t-butyl))1-CO- (CH2)18-CO2-(t-butyl).
  MOD_RES 10: note = The sidechain of glutamine is protected by a Trityl (Trt) protecting group.
  MOD_RES 11: note = The sidechain of Tryptophan is protected by a t-butyloxycarbonyl (Boc) protecting group.
  MOD_RES 18: note = The sidechain of serine is protected by t-butyl.
  MOD_RES 19: note = The sidechain of serine is protected by t-butyl.
  MOD_RES 25: note = The sidechain of serine is protected by t-butyl.
  MOD_RES 25: note = Serine at position 25 is amidated as a C-terminal primary amide.
DKIAQKAFVQWLIAGGPSSGAPPPS

SEQ ID NO: 22 - protein, 39 aa, synthetic construct; identical to SEQ ID NO: 1
  REGION 1..39: note = Synthetic Construct
  MOD_RES 1: note = N-terminus is protected by (t-butyloxycarbonyl) Boc.
  MOD_RES 1: note = The sidechain of tyrosine is protected by t-butyl.
  MOD_RES 2: note = Xaa at position 2 is 2-Aminoisobutyric Acid (Aib).
  MOD_RES 3: note = The sidechain of glutamic acid is protected by t-butyl.
  MOD_RES 5: note = The sidechain of threonine is protected by t-butyl.
  MOD_RES 7: note = The sidechain of threonine is protected by t-butyl.
  MOD_RES 8: note = The sidechain of serine is protected by t-butyl.
  MOD_RES 9: note = The sidechain of aspartic acid is protected by t-butyl.
  MOD_RES 10: note = The sidechain of tyrosine is protected by t-butyl.
  MOD_RES 11: note = The sidechain of serine is protected by t-butyl.
  MOD_RES 13: note = Xaa at position 13 is 2-Aminoisobutyric Acid (Aib).
  MOD_RES 15: note = The sidechain of aspartic acid is protected by t-butyl.
  MOD_RES 16: note = The sidechain of lysine is protected by a t-butyloxycarbonyl (Boc) protecting group.
  MOD_RES 19: note = The sidechain of glutamine is protected by a Trityl (Trt) protecting group.
  MOD_RES 20: note = Lys at position 20 is chemically modified through conjugation to the epsilon-amino group of the K side-chain with (2-[2-(2-Amino-ethoxy)-ethoxy]-acetyl)2-(gamma-Glu(t-butyl))1-CO- (CH2)18-CO2-(t-butyl).
  MOD_RES 24: note = The sidechain of glutamine is protected by a Trityl (Trt) protecting group.
  MOD_RES 25: note = The sidechain of Tryptophan is protected by a t-butyloxycarbonyl (Boc) protecting group.
  MOD_RES 32: note = The sidechain of serine is protected by t-butyl.
  MOD_RES 33: note = The sidechain of serine is protected by t-butyl.
  MOD_RES 39: note = The sidechain of serine is protected by t-butyl.
  MOD_RES 39: note = Serine at position 39 is amidated as a C-terminal primary amide.

SEQ ID NO: 23 - protein, 39 aa, synthetic construct; identical to SEQ ID NO: 1
  REGION 1..39: note = Synthetic Construct
  MOD_RES 1: note = N-terminus is protected by (t-butyloxycarbonyl) Boc.
  MOD_RES 1: note = The sidechain of tyrosine is protected by t-butyl.
  MOD_RES 2: note = Xaa at position 2 is 2-Aminoisobutyric Acid (Aib).
  MOD_RES 3: note = The sidechain of glutamic acid is protected by t-butyl.
  MOD_RES 5: note = The sidechain of threonine is protected by t-butyl.
  MOD_RES 7: note = The sidechain of threonine is protected by t-butyl.
  MOD_RES 8: note = The sidechain of serine is protected by t-butyl.
  MOD_RES 9: note = The sidechain of aspartic acid is protected by t-butyl.
  MOD_RES 10: note = The sidechain of tyrosine is protected by t-butyl.
  MOD_RES 11: note = The sidechain of serine is protected by t-butyl.
  MOD_RES 13: note = Xaa at position 13 is 2-Aminoisobutyric Acid (Aib).
  MOD_RES 15: note = The sidechain of aspartic acid is protected by t-butyl.
  MOD_RES 16: note = The sidechain of lysine is protected by a t-butyloxycarbonyl (Boc) protecting group.
  MOD_RES 19: note = The sidechain of glutamine is protected by a Trityl (Trt) protecting group.
  MOD_RES 20: note = The epsilon amino group of K is modified with 5,5-dimethyl-2-(3-methylbutylidene)cyclohexane-1,3-dione
  MOD_RES 24: note = The sidechain of glutamine is protected by a Trityl (Trt) protecting group.
  MOD_RES 25: note = The sidechain of Tryptophan is protected by a t-butyloxycarbonyl (Boc) protecting group.
  MOD_RES 32: note = The sidechain of serine is protected by t-butyl.
  MOD_RES 33: note = The sidechain of serine is protected by t-butyl.
  MOD_RES 39: note = The sidechain of serine is protected by t-butyl.
  MOD_RES 39: note = The C-terminal serine is amidated and is bound to Sieber resin through this amine group.

SEQ ID NO: 24 - protein, 39 aa, synthetic construct; identical to SEQ ID NO: 1
  REGION 1..39: note = Synthetic Construct
  MOD_RES 1: note = N-terminus is protected by (t-butyloxycarbonyl) Boc.
  MOD_RES 1: note = The sidechain of tyrosine is protected by t-butyl.
  MOD_RES 2: note = Xaa at position 2 is 2-Aminoisobutyric Acid (Aib).
  MOD_RES 3: note = The sidechain of glutamic acid is protected by t-butyl.
  MOD_RES 5: note = The sidechain of threonine is protected by t-butyl.
  MOD_RES 7: note = The sidechain of threonine is protected by t-butyl.
  MOD_RES 8: note = The sidechain of serine is protected by t-butyl.
  MOD_RES 9: note = The sidechain of aspartic acid is protected by t-butyl.
  MOD_RES 10: note = The sidechain of tyrosine is protected by t-butyl.
  MOD_RES 11: note = The sidechain of serine is protected by t-butyl.
  MOD_RES 13: note = Xaa at position 13 is 2-Aminoisobutyric Acid (Aib).
  MOD_RES 15: note = The sidechain of aspartic acid is protected by t-butyl.
  MOD_RES 16: note = The sidechain of lysine is protected by a t-butyloxycarbonyl (Boc) protecting group.
  MOD_RES 19: note = The sidechain of glutamine is protected by a Trityl (Trt) protecting group.
  MOD_RES 24: note = The sidechain of glutamine is protected by a Trityl (Trt) protecting group.
  MOD_RES 25: note = The sidechain of Tryptophan is protected by a t-butyloxycarbonyl (Boc) protecting group.
  MOD_RES 32: note = The sidechain of serine is protected by t-butyl.
  MOD_RES 33: note = The sidechain of serine is protected by t-butyl.
  MOD_RES 39: note = The sidechain of serine is protected by t-butyl.
  MOD_RES 39: note = The C-terminal serine is amidated and is bound to Sieber resin through this amine group.

SEQ ID NO: 25 - protein, 10 aa, synthetic construct
  REGION 1..10: note = Synthetic Construct
  MOD_RES 3: note = The sidechain of serine is protected by t-butyl.
  MOD_RES 4: note = The sidechain of serine is protected by t-butyl.
  MOD_RES 10: note = The sidechain of serine is protected by t-butyl.
  MOD_RES 10: note = Serine at position 10 is amidated as a C-terminal primary amide.
GPSSGAPPPS

SEQ ID NO: 26 - protein, 8 aa, synthetic construct
  REGION 1..8: note = Synthetic Construct
  MOD_RES 1: note = N-terminus is protected by Fmoc.
  MOD_RES 3: note = The sidechain of glutamine is protected by a Trityl (Trt) protecting group.
  MOD_RES 4: note = The sidechain of Tryptophan is protected by a t-butyloxycarbonyl (Boc) protecting group.
FVQWLIAG

SEQ ID NO: 27 - protein, 18 aa, synthetic construct
  REGION 1..18: note = Synthetic Construct
  MOD_RES 3: note = The sidechain of glutamine is protected by a Trityl (Trt) protecting group.
  MOD_RES 4: note = The sidechain of Tryptophan is protected by a t-butyloxycarbonyl (Boc) protecting group.
  MOD_RES 11: note = The sidechain of serine is protected by t-butyl.
  MOD_RES 12: note = The sidechain of serine is protected by t-butyl.
  MOD_RES 18: note = The sidechain of serine is protected by t-butyl.
  MOD_RES 18: note = Serine at position 18 is amidated as a C-terminal primary amide.
FVQWLIAGGPSSGAPPPS

SEQ ID NO: 28 - protein, 7 aa, synthetic construct
  REGION 1..7: note = Synthetic Construct
  MOD_RES 1: note = N-terminus is protected by Fmoc.
  MOD_RES 1: note = The sidechain of aspartic acid is protected by t-butyl.
  MOD_RES 2: note = The sidechain of lysine is protected by a t-butyloxycarbonyl (Boc) protecting group.
  MOD_RES 5: note = The sidechain of glutamine is protected by a Trityl (Trt) protecting group.
  MOD_RES 6: note = Lys at position 6 is chemically modified through conjugation to the epsilon-amino group of the K side-chain with (2-[2-(2-Amino-ethoxy)-ethoxy]-acetyl)2-(gamma-Glu(t-butyl))1-CO- (CH2)18-CO2-(t-butyl).
DKIAQKA

SEQ ID NO: 29 - protein, 25 aa, synthetic construct
  REGION 1..25: note = Synthetic Construct
  MOD_RES 1: note = The sidechain of aspartic acid is protected by t-butyl.
  MOD_RES 2: note = The sidechain of lysine is protected by a t-butyloxycarbonyl (Boc) protecting group.
  MOD_RES 5: note = The sidechain of glutamine is protected by a Trityl (Trt) protecting group.
  MOD_RES 6: note = Lys at position 6 is chemically modified through conjugation to the epsilon-amino group of the K side-chain with (2-[2-(2-Amino-ethoxy)-ethoxy]-acetyl)2-(gamma-Glu(t-butyl))1-CO- (CH2)18-CO2-(t-butyl).
  MOD_RES 10: note = The sidechain of glutamine is protected by a Trityl (Trt) protecting group.
  MOD_RES 11: note = The sidechain of Tryptophan is protected by a t-butyloxycarbonyl (Boc) protecting group.
  MOD_RES 18: note = The sidechain of serine is protected by t-butyl.
  MOD_RES 19: note = The sidechain of serine is protected by t-butyl.
  MOD_RES 25: note = The sidechain of serine is protected by t-butyl.
  MOD_RES 25: note = Serine at position 25 is amidated as a C-terminal primary amide.
DKIAQKAFVQWLIAGGPSSGAPPPS

SEQ ID NO: 30 - protein, 14 aa, synthetic construct
  REGION 1..14: note = Synthetic Construct
  MOD_RES 1: note = N-terminus is protected by (t-butyloxycarbonyl) Boc.
  MOD_RES 1: note = The sidechain of tyrosine is protected by t-butyl.
  MOD_RES 2: note = Xaa at position 2 is 2-Aminoisobutyric Acid (Aib).
  MOD_RES 3: note = The sidechain of glutamic acid is protected by t-butyl.
  MOD_RES 5: note = The sidechain of threonine is protected by t-butyl.
  MOD_RES 7: note = The sidechain of threonine is protected by t-butyl.
  MOD_RES 8: note = The sidechain of serine is protected by t-butyl.
  MOD_RES 9: note = The sidechain of aspartic acid is protected by t-butyl.
  MOD_RES 10: note = The sidechain of tyrosine is protected by t-butyl.
  MOD_RES 11: note = The sidechain of serine is protected by t-butyl.
  MOD_RES 13: note = Xaa at position 13 is 2-Aminoisobutyric Acid (Aib).
YXEGTFTSDYSIXL

SEQ ID NO: 31 - protein, 39 aa, synthetic construct; identical to SEQ ID NO: 1
  REGION 1..39: note = Synthetic Construct
  MOD_RES 1: note = N-terminus is protected by (t-butyloxycarbonyl) Boc.
  MOD_RES 1: note = The sidechain of tyrosine is protected by t-butyl.
  MOD_RES 2: note = Xaa at position 2 is 2-Aminoisobutyric Acid (Aib).
  MOD_RES 3: note = The sidechain of glutamic acid is protected by t-butyl.
  MOD_RES 5: note = The sidechain of threonine is protected by t-butyl.
  MOD_RES 7: note = The sidechain of threonine is protected by t-butyl.
  MOD_RES 8: note = The sidechain of serine is protected by t-butyl.
  MOD_RES 9: note = The sidechain of aspartic acid is protected by t-butyl.
  MOD_RES 10: note = The sidechain of tyrosine is protected by t-butyl.
  MOD_RES 11: note = The sidechain of serine is protected by t-butyl.
  MOD_RES 13: note = Xaa at position 13 is 2-Aminoisobutyric Acid (Aib).
  MOD_RES 15: note = The sidechain of aspartic acid is protected by t-butyl.
  MOD_RES 16: note = The sidechain of lysine is protected by a t-butyloxycarbonyl (Boc) protecting group.
  MOD_RES 19: note = The sidechain of glutamine is protected by a Trityl (Trt) protecting group.
  MOD_RES 20: note = Lys at position 20 is chemically modified through conjugation to the epsilon-amino group of the K side-chain with (2-[2-(2-Amino-ethoxy)-ethoxy]-acetyl)2-(gamma-Glu(t-butyl))1-CO- (CH2)18-CO2-(t-butyl).
  MOD_RES 24: note = The sidechain of glutamine is protected by a Trityl (Trt) protecting group.
  MOD_RES 25: note = The sidechain of Tryptophan is protected by a t-butyloxycarbonyl (Boc) protecting group.
  MOD_RES 32: note = The sidechain of serine is protected by t-butyl.
  MOD_RES 33: note = The sidechain of serine is protected by t-butyl.
  MOD_RES 39: note = The sidechain of serine is protected by t-butyl.
  MOD_RES 39: note = Serine at position 39 is amidated as a C-terminal primary amide.

SEQ ID NO: 32 - protein, 17 aa, synthetic construct
  REGION 1..17: note = Synthetic Construct
  SITE 2: note = MISC_FEATURE - Xaa at position 2 is Aib
  SITE 13: note = MISC_FEATURE - Xaa at position 13 is Aib
  MOD_RES 17: note = The C-terminal hydroxyl of Isoleucine is modified with hydrazide (N-NH2)
YXEGTFTSDYSIXLDKI

SEQ ID NO: 33 - protein, 22 aa, synthetic construct
  REGION 1..22: note = Synthetic Construct
  MOD_RES 3: note = Lys at position 3 is chemically modified through conjugation to the epsilon-amino group of the K side-chain with (2-[2-(2-Amino-ethoxy)-ethoxy]-acetyl)2-(gamma-Glu)1-CO-(CH2)18-C O2H
  MOD_RES 22: note = Ser at position 22 is amidated as a C-terminal primary amide
CQKAFVQWLIAGGPSSGAPPPS

SEQ ID NO: 34 - protein, 17 aa, synthetic construct
  REGION 1..17: note = Synthetic Construct
  SITE 2: note = MISC_FEATURE - Xaa at position 2 is Aib
  SITE 13: note = MISC_FEATURE - Xaa at position 13 is Aib
  MOD_RES 17: note = The C terminal hydroxyl is modified with S-CH2-CF3
YXEGTFTSDYSIXLDKI

SEQ ID NO: 35 - protein, 39 aa, synthetic construct
  REGION 1..39: note = Synthetic Construct
  SITE 2: note = MISC_FEATURE - Xaa at position 2 is Aib
  SITE 13: note = MISC_FEATURE - Xaa at position 13 is Aib
  MOD_RES 20: note = Lys at position 20 is chemically modified through conjugation to the epsilon-amino group of the K side-chain with (2-[2-(2-Amino-ethoxy)-ethoxy]-acetyl)2-(gamma-Glu)1-CO-(CH2)18-C O2H
  MOD_RES 39: note = Ser at position 39 is amidated as a C-terminal primary amide
YXEGTFTSDYSIXLDKICQKAFVQWLIAGGPSSGAPPPS

SEQ ID NO: 36 - protein, 20 aa, synthetic construct
  REGION 1..20: note = Synthetic Construct
  SITE 2: note = MISC_FEATURE - Xaa at position 2 is Aib
  SITE 13: note = MISC_FEATURE - Xaa at position 13 is Aib
  MOD_RES 20: note = Lys at position 20 is chemically modified through conjugation to the epsilon-amino group of the K side-chain with (2-[2-(2-Amino-ethoxy)-ethoxy]-acetyl)2-(gamma-Glu)1-CO-(CH2)18-C O2H
  MOD_RES 20: note = The C-terminal hydroxyl is modified with hydrazide (-N-NH2)
YXEGTFTSDYSIXLDKIAQK

SEQ ID NO: 37 - protein, 19 aa, synthetic construct
  REGION 1..19: note = Synthetic Construct
  MOD_RES 19: note = Ser at position 19 is amidated as a C-terminal primary amide
CFVQWLIAGGPSSGAPPPS

SEQ ID NO: 38 - protein, 20 aa, synthetic construct
  REGION 1..20: note = Synthetic Construct
  SITE 2: note = MISC_FEATURE - Xaa at position 2 is Aib
  SITE 13: note = MISC_FEATURE - Xaa at position 13 is Aib
  MOD_RES 20: note = Lys at position 20 is chemically modified through conjugation to the epsilon-amino group of the K side-chain with (2-[2-(2-Amino-ethoxy)-ethoxy]-acetyl)2-(gamma-Glu)1-CO-(CH2)18-C O2H
  MOD_RES 20: note = The C-terminal hydroxyl is modified with 4-mercaptophenylacetic acid
YXEGTFTSDYSIXLDKIAQK

SEQ ID NO: 39 - protein, 39 aa, synthetic construct
  REGION 1..39: note = Synthetic Construct
  SITE 2: note = MISC_FEATURE - Xaa at position 2 is is nonnaturally occurring amino acid 2-Aminoisobutyric Acid
  SITE 13: note = MISC_FEATURE - Xaa at position 13 is is nonnaturally occurring amino acid 2-Aminoisobutyric Acid
  MOD_RES 20: note = Lys at position 20 is chemically modified through conjugation to the epsilon-amino group of the K side-chain with (2-[2-(2-Amino-ethoxy)-ethoxy]-acetyl)2-(gamma-Glu)1-CO-(CH2)18-C O2H
  MOD_RES 39: note = Ser at position 39 is amidated as a C-terminal primary amide
YXEGTFTSDYSIXLDKIAQKCFVQWLIAGGPSSGAPPPS

SEQ ID NO: 40 - protein, 39 aa, synthetic construct
  REGION 1..39: note = Synthetic Construct
  SITE 2: note = MISC_FEATURE - Xaa at position 2 is Aib
  MOD_RES 7..8: note = Thr at position 7 and Ser at position 8 form a depsi peptide
  SITE 13: note = MISC_FEATURE - Xaa at position 13 is Aib
  MOD_RES 20: note = Lys at position 20 is chemically modified through conjugation to the epsilon-amino group of the K side-chain with (2-[2-(2-Amino-ethoxy)-ethoxy]-acetyl)2-(gamma-Glu)1-CO-(CH2)18-C O2H
  MOD_RES 39: note = Ser at position 39 is amidated as a C-terminal primary amide
YXEGTFXXDYSIXLDKIAQKAFVQWLIAGGPSSGAPPPS